European Patent Application EP 4 159 850 A1, published April 5, 2023. Title: Production of desaturated fatty alcohols and desaturated fatty acyl acetates in yeast. Applicant: Danmarks Tekniske Universitet. The sequence listing filed with the application follows.

SEQUENCE LISTING (74 sequences)

SEQ ID NO: 1 - DNA, 1107 bp, synthetic construct
  misc_feature 1..1107: note = codon-optimized nucleotide sequence
  misc_feature 1..1107: note = Y.lipolytica codon-optimized nucleotide sequence of delta9desaturase from Pelargonium hortorum
  source 1..1107: mol_type = other DNA
atgggcgtgctgctgaacatctgttcgtctcccttccccgtggtggcctctgccgcctctacctctatctctaaggtgaaccacatccgaaaggtgggcgtgaccggcgtgatggctccccagaagatcgagatcttcaagtctatggaggagtggggcaagcacaacatcctgcccctggccaagcccgtcgagaagtcttggcagcctaccgacttcctgcccgacccctcgtctgagggcttcatggaggagtacaacgccttcaaggagcgaactcgagagctgcccgacgagtacttcgtggtgctggccggcgacatgatcaccgaggaggccctgcccacctaccagaccctggtgaaccgacccgacgaggtggccgacgagactggccactctgagtctccctgggccgtgtggtcccgagcctggaccgccgaggagaaccgacacggcgacctgctgaacaagtacctgtacctgtctggcaagctggacatgcgacaggtcgagaagaccatccagtacctgatcgctctgggccaggacatcggcaccgagaagaacccctaccacctgttcatctacacctcgttccaggagcgagccaccttcatctctcacgccaacaccgccaagctggcccagcagcacggcgacaagcagctggctcagatctgcggcaccattgccgccgacgagaagcgacatgagactgcctacacccgaatcgtggacaagctgttcgagctggaccccgacgagactatgtcttgcctggcccacatgatgaagcgaaagatcaccatgcccgcccacctgatgcgagatggccgagatccccacctgttccagcacttctctgtggtggcctcccgaaccggcgtgtacaccgtgatggactacatcaacatcctcgagcacttcgtcgagaagtggaacatcgagaagatcaccgccggactgtctgacaagggccgagaggcccaggactacgtgtgcaagctgggcgagcgactgcgaaaggtcgaggagcgagctcatcagcgagtggtgcaggccgaccccatccccttctcttggatcttcgaccgaaaggtgtaa

SEQ ID NO: 2 - protein, 368 aa, Pelargonium x hortorum
MGVLLNICSSPFPVVASAASTSISKVNHIRKVGVTGVMAPQKIEIFKSMEEWGKHNILPLAKPVEKSWQPTDFLPDPSSEGFMEEYNAFKERTRELPDEYFVVLAGDMITEEALPTYQTLVNRPDEVADETGHSESPWAVWSRAWTAEENRHGDLLNKYLYLSGKLDMRQVEKTIQYLIALGQDIGTEKNPYHLFIYTSFQERATFISHANTAKLAQQHGDKQLAQICGTIAADEKRHETAYTRIVDKLFELDPDETMSCLAHMMKRKITMPAHLMRDGRDPHLFQHFSVVASRTGVYTVMDYINILEHFVEKWNIEKITAGLSDKGREAQDYVCKLGERLRKVEERAHQRVVQADPIPFSWIFDRKV

SEQ ID NO: 3 - DNA, 1191 bp, synthetic construct
  misc_feature 1..1191: note = codon-optimized nucleotide sequence
  misc_feature 1..1191: note = Y.lipolytica codon-optimized nucleotide sequence of delta9desaturase from Ricinus communis
  source 1..1191: mol_type = other DNA
atggccctgaagctgaaccccttcctgtctcaaacccagaagctgccctctttcgccctgcctcccatggcctctacccgatctcccaagttctacatggcctccaccctgaagtctggctctaaggaggtcgagaacctgaagaagcccttcatgcctccccgagaggtgcacgtgcaggtcacccactctatgcctccccagaagatcgagatcttcaagtctctggacaactgggccgaggagaacatcctggtccacctgaagcccgtcgagaagtgctggcagccccaggacttcctgcccgaccccgcctctgacggcttcgacgagcaggtccgagagctgcgagagcgagccaaggagatccccgacgactacttcgtggtgctggtgggcgacatgatcaccgaggaggccctgcccacctaccagaccgccctgaaccgaggcgacggcgtgcgagatgagactggcgcctctcccacctcttgggccatctggacccgagcctggaccgctgaggagaaccgacacggcgacctgctgaacaagtacctgtacctgtctggccgagtggacatgcgacagatcgagaagaccatccagtacctgatcggctctggcatggacgtgcgagtcgagaactctccctacctgctgttcatctacacctcgttccaggagcgagccaccttcatctctcacggcaacaccgcccgacaggccaaggagcacggcgacatcaagctggcccagatctgcggcaccattgccgccgacgagaagcgacacgagactgcctacaccaagatcgtcgagaagctgttcgagatcgaccccgacggcaccgtgctggccttcgccgacatgatgcgaaagaagatctctatgcccgcccacctgatgtacgacggccgagatgacaacctgttcgaccacttctctgccgtggctcagcgactgggcgtgtacaccgccaaggactacgccgacatcctcgagtttctggtgggccgatggaaggtggacaagctgaccggcctgtctgccgagggccagaaggcccaggactacgtctgccgactgcctccccgaatccgacgactcgaggagcgagctcagggccgagctaaggaggctcccaccatgcccttctcttggatcttcgaccgacaggtgaagctgtaa

SEQ ID NO: 4 - protein, 396 aa, Ricinus communis
MALKLNPFLSQTQKLPSFALPPMASTRSPKFYMASTLKSGSKEVENLKKPFMPPREVHVQVTHSMPPQKIEIFKSLDNWAEENILVHLKPVEKCWQPQDFLPDPASDGFDEQVRELRERAKEIPDDYFVVLVGDMITEEALPTYQTALNRGDGVRDETGASPTSWAIWTRAWTAEENRHGDLLNKYLYLSGRVDMRQIEKTIQYLIGSGMDVRVENSPYLLFIYTSFQERATFISHGNTARQAKEHGDIKLAQICGTIAADEKRHETAYTKIVEKLFEIDPDGTVLAFADMMRKKISMPAHLMYDGRDDNLFDHFSAVAQRLGVYTAKDYADILEFLVGRWKVDKLTGLSAEGQKAQDYVCRLPPRIRRLEERAQGRAKEAPTMPFSWIFDRQVKL

SEQ ID NO: 5 - DNA, 1059 bp, synthetic construct
  misc_feature 1..1059: note = codon-optimized nucleotide sequence
  misc_feature 1..1059: note = S. cerevisiae codon-optimized nucleotide sequence of delta9desaturase from Amyelois transitella Atr236
  source 1..1059: mol_type = other DNA
atgccgcctcagggtcaagatcgcgagtcctgggttctgtacgagaccgacgacaagacgcaagatggtggcactcacgtggtgcctccctccgccgagaaaagagtgtggaaaatcgtctggaggaatgtcatcgcatttgctctgctccacatcggaggcgtttacggcgcttatttgttcctcttcaaagctatgtggctgaccgatttgtttgcggtatttctgtacctgtgctccggcctgggcgtcactgcgggcgcgcaccggctgtgggcacacaagtcgtacaaggcgcggctgcctctccgcctgttgcttactgtcttcaacaccatagcttttcaggatgccgtgatcgactgggctcgcgaccaccgcctgcaccataagtactcggagacggacgccgatccccacaacgcaacaagggggttcttcttctcccacattggctggttgctcgtcaggaaacacccacaaatcaaggagaaagggcccaccatcgacctgaacgacttgagggccgatcccgtactccacttccagaagaaatactatttataccttatgcccttggcatgtttcgtcatgcccacattagtacctacactctggggtgaatctctatggaacgcgtatttcgtatgcgctatcttcagatacatatatgttctaaacgtcacttggctcgtaaactcagctgcgcacgcttggggaagcaaaccgtacgacaaaaacatcaaccctgtggaaaccaagcctgtatccttggtggtccttggagaaggcttccacaattaccaccacactttcccgtgggattacaagactgccgaattaggagattactctttaaacttctccaaattattcatcgatgctatggcaaaaataggttgggcttatgacctgaaaacggtctctcctgatgtgatcgagaagcgtgtgaagaggacgggagacggcagtcaccacgtctggggctgggacgacaaagacgtcccggttgaagaaaaagaagaagccaccatctttaacccttcgaaagatgaataa

SEQ ID NO: 6 - protein, 352 aa, Amyelois transitella
MPPQGQDRESWVLYETDDKTQDGGTHVVPPSAEKRVWKIVWRNVIAFALLHIGGVYGAYLFLFKAMWLTDLFAVFLYLCSGLGVTAGAHRLWAHKSYKARLPLRLLLTVFNTIAFQDAVIDWARDHRLHHKYSETDADPHNATRGFFFSHIGWLLVRKHPQIKEKGPTIDLNDLRADPVLHFQKKYYLYLMPLACFVMPTLVPTLWGESLWNAYFVCAIFRYIYVLNVTWLVNSAAHAWGSKPYDKNINPVETKPVSLVVLGEGFHNYHHTFPWDYKTAELGDYSLNFSKLFIDAMAKIGWAYDLKTVSPDVIEKRVKRTGDGSHHVWGWDDKDVPVEEKEEATIFNPSKDE

SEQ ID NO: 7 - DNA, 1059 bp, synthetic construct
  misc_feature 1..1059: note = codon-optimized nucleotide sequence
  misc_feature 1..1059: note = S. cerevisiae codon-optimized nucleotide sequence of delta9desaturase from Amyelois transitella Atr1432
  source 1..1059: mol_type = other DNA
atggctccaaatgccacagatgctaatggggttctgtttgagacggatgcagctaccccagacctggccctacctcacgcccctgtacagcaagcggacaattaccctaaaaaatatgtgtggagaaatataatattatttgcctatctccacattgctgcactctatggtggctacttgttcttgttccatgctaaatggcagacagatatatttgcttacattctgtatgtgatgtcaggcttgggaataacggcaggagcccatcgtctgtgggcccacaagtcctacaaagctaaatggccactcagattgatacttgtcatctttaacactctggcattccaggactctgcaatcgactggtctcgcgaccaccgaatgcaccacaaatactcggaaactgatgctgatccccacaacgcgacccgcggtttcttcttctcccacattggctggctgctggttaggaagcaccctgaacttaagaggaaaggcaaaggtctggaccttagtgacttatatgctgaccccattttgagattccaaaagaagtactacttgatcctgatgcccctcacttgcttcgtgttacctacggtcatccccgtgtattactggggcgagacttggaccaacgccttcttcgtggccgctcttttccggtatgccttcatccttaacgtcacctggctggtcaattctgctgctcacaagtggggcgataagccttacgatagaaacatcaagccttcggaaaatatttccgtctccatgttcgcgctcggagaaggcttccacaactaccaccatactttcccctgggactacaagaccgcggaacttggcaacaacatgctcaatttcacgactaacttcatcaatttctttgctaaaatcggttgggcgtacgatctgaaaactgtttccgatgaaattgttaggagccgcgctaagagaacaggagatggttctcaccatctatggggctggggtgataaggatcactctcgtgaggaaatggccgccgctataaggatacacccgaaagatgactag

SEQ ID NO: 8 - protein, 352 aa, Amyelois transitella
MAPNATDANGVLFETDAATPDLALPHAPVQQADNYPKKYVWRNIILFAYLHIAALYGGYLFLFHAKWQTDIFAYILYVMSGLGITAGAHRLWAHKSYKAKWPLRLILVIFNTLAFQDSAIDWSRDHRMHHKYSETDADPHNATRGFFFSHIGWLLVRKHPELKRKGKGLDLSDLYADPILRFQKKYYLILMPLTCFVLPTVIPVYYWGETWTNAFFVAALFRYAFILNVTWLVNSAAHKWGDKPYDRNIKPSENISVSMFALGEGFHNYHHTFPWDYKTAELGNNMLNFTTNFINFFAKIGWAYDLKTVSDEIVRSRAKRTGDGSHHLWGWGDKDHSREEMAAAIRIHPKDD

SEQ ID NO: 9 - DNA, 1086 bp, synthetic construct
  misc_feature 1..1086: note = codon-optimized nucleotide sequence
  misc_feature 1..1086: note = S. cerevisiae codon-optimized nucleotide sequence of delta9desaturase from Drosophila melanogaster Dmd9
  source 1..1086: mol_type = other DNA
atggctccatactctagaatctaccaccaagataagtcctctagagaaactggtgttttgttcgaagatgatgctcaaaccgttgattctgatttgactaccgatagattccaattgaagagagccgaaaaaagaagattgccattggtttggagaaacatcatcttgttcgctttggttcatttggctgccttgtatggtttacattccattttcactagagctaagttggctactactttgtttgctgctggtttgtacattatcggtatgttgggtgttactgctggtgctcatagattgtgggctcatagaacttacaaagctaaatggcctttgagattgttgttggtcatcttcaacaccattgctttccaagatgctgtttatcattgggccagagatcatagagttcatcacaaatactctgaaaccgatgctgatccacataatgctactagaggtttcttcttctctcatgttggttggttgttgtgcaagaaacacccagatatcaaagaaaagggtagaggtttggatttgtccgatttgagagctgatccaatcttgatgtttcaaagaaagcactactacatcttgatgccattggcttgttttgttttgccaaccgttattccaatggtctactggaacgaaactttggcttcttcttggtttgttgctactatgttcagatggtgcttccaattgaatatgacctggttggttaattccgctgctcataagtttggtaatagaccatacgataagaccatgaacccaactcaaaatgctttcgtttctgctttcacttttggtgaaggttggcataattaccatcatgcttttccatgggattacaagactgctgaatggggttgttactctttgaacattactaccgccttcattgatttgttcgctaaaattggttgggcctacgatttgaaaactgttgctccagatgttatccaaagaagagttttgagaactggtgatggttctcatgaattgtggggttggggtgataaggatttgaccgctgaagatgctagaaacgttttgttggttgacaagtccagataa

SEQ ID NO: 10 - protein, 361 aa, Drosophila melanogaster
MAPYSRIYHQDKSSRETGVLFEDDAQTVDSDLTTDRFQLKRAEKRRLPLVWRNIILFALVHLAALYGLHSIFTRAKLATTLFAAGLYIIGMLGVTAGAHRLWAHRTYKAKWPLRLLLVIFNTIAFQDAVYHWARDHRVHHKYSETDADPHNATRGFFFSHVGWLLCKKHPDIKEKGRGLDLSDLRADPILMFQRKHYYILMPLACFVLPTVIPMVYWNETLASSWFVATMFRWCFQLNMTWLVNSAAHKFGNRPYDKTMNPTQNAFVSAFTFGEGWHNYHHAFPWDYKTAEWGCYSLNITTAFIDLFAKIGWAYDLKTVAPDVIQRRVLRTGDGSHELWGWGDKDLTAEDARNVLLVDKSR

SEQ ID NO: 11 - DNA, 1062 bp, synthetic construct
  misc_feature 1..1062: note = codon-optimized nucleotide sequence
  misc_feature 1..1062: note = Y. lipolytica codon-optimized nucleotide sequence of delta9desaturase from Spodoptera litura Des11
  source 1..1062: mol_type = other DNA
atggctcccaacatctctgaggacgtgaacggcgtgctgttcgagtctgacgccgctactcccgacctggctctggcccgacctcctgtgcagaaggccgacaacaagcccaagcagctggtgtggcgaaacatcatcctgttcgcctacctgcacctggccgctctgtacggcggctacctgttcctgttctctgccaagtggcagaccgacatcttcgcctacatcctgtacgtgatctctggcctgggcatcaccgctggcgcccaccgactgtgggctcacaagtcttacaaggctaagtggcccctgaaggtgatcctgatcatcttcaacaccgtggccttccaggacgccgccatggactgggcccgagatcaccgaatgcaccacaagtactctgagactgacgctgaccctcacaacgctacccgaggcttcttcttctctcacatcggctggctgctggtgcgaaagcaccccgacctgaaggaaaagggcaagggcctcgacatgtctgacctgctggctgaccccgtgctgcgattccagaagaagtactacctgctgctgatgcccctggcctgcttcgtcatgcccaccgtgattcccgtgtacctgtggggcgagacttggaccaacgccttcttcgtggccgccatgttccgatacgccttcattctgaacgtgacctggctggtgaactctgctgcccacaagtggggcgacaagccctacgacaagtctatcaagccctctgagaacatgtctgtggccatgttcgccctcggcgagggattccacaactaccaccacacattcccttgggactacaagaccgccgagttcggcaacaacaagctgaacttcactaccgccttcatcaactttttcgccaagatcggctgggcttacgacatgaagaccgtgtctgaggacatcgtgaagaaccgagtgaagcgaaccggcgacggctctcaccacctctggggctggggcgacgagaaccagcctaaggaagagatcgaggccgccatccgaatcaaccccaaggacgactaa

SEQ ID NO: 12 - protein, 353 aa, Spodoptera litura
MAPNISEDVNGVLFESDAATPDLALARPPVQKADNKPKQLVWRNIILFAYLHLAALYGGYLFLFSAKWQTDIFAYILYVISGLGITAGAHRLWAHKSYKAKWPLKVILIIFNTVAFQDAAMDWARDHRMHHKYSETDADPHNATRGFFFSHIGWLLVRKHPDLKEKGKGLDMSDLLADPVLRFQKKYYLLLMPLACFVMPTVIPVYLWGETWTNAFFVAAMFRYAFILNVTWLVNSAAHKWGDKPYDKSIKPSENMSVAMFALGEGFHNYHHTFPWDYKTAEFGNNKLNFTTAFINFFAKIGWAYDMKTVSEDIVKNRVKRTGDGSHHLWGWGDENQPKEEIEAAIRINPKDD

SEQ ID NO: 13 - DNA, 1050 bp, synthetic construct
  misc_feature 1..1050: note = codon-optimized nucleotide sequence
  misc_feature 1..1050: note = Y.lipolytica codon-optimized nucleotide sequence of delta 9desaturase from Chauliognathus lugubris Cld9
  source 1..1050: mol_type = other DNA
atggctcccaactctaacgacgccaccggcgtgctgcaagagactgacgacgacgtgtcctctaaccaggtcctgcagcagatcaccaagtctgagaagtctaagctgatcatcgtgtggtctaacgtgatgtacttcgtgatcctgcacgtgggcgccctgtacggcctgtggctgctgctgacctctgctcagatctggacctgcctgtgggtgttcgccatgtacgagttcggcgagatctgcatcaccgctggcgtgcaccgactgtggtcccaccgatcttacaaggccaagtggcccctgcgactgttccacaccatgggacagaccctggccttccaggacgccgtggtggactgggcccgagatcaccgagtgcaccacaagtactctgaaaccgacgctgaccctcacaacgccaagcgaggcttcttcttctctcacatgggctggctgatgtgccgaaagtccaagcaggtcaaggaaaagggcaaggaacccgacatctctgacctgtacgctgatcccatcctgcgataccaaaagaagtactacatgctgttcatgcccctgatgtgcttcgctttccccaccgtggtgcccctgtacttctggaacgagtctctcaagaccgccttcttcgtgaacatcttccggtacatcttctccctgcacgccacctggctggtgaactctgccgctcacctctacggcgagaagccctacaacaagcacattaaccccgccgagaacctggccgtgtctctgatcgtgaacggcgaacgatggcacaactaccaccacacattcccttgggactacaaggccggcgagttcggacgatacggcaccaacctgaccaccgtgttcatcaacgccatggccaagatcggcctggcctacgacctgaagttcgtgcccgaggacgtggtgaagcgacgagtgcacaagaccggcgacggctctcacgccgtgtggggctggggcgacaaggaccagaccgtggaagagatttctaagaccatcgtggcctacaaccagtcttaa

SEQ ID NO: 14 - protein, 349 aa, Chauliognathus lugubris
MAPNSNDATGVLQETDDDVSSNQVLQQITKSEKSKLIIVWSNVMYFVILHVGALYGLWLLLTSAQIWTCLWVFAMYEFGEICITAGVHRLWSHRSYKAKWPLRLFHTMGQTLAFQDAVVDWARDHRVHHKYSETDADPHNAKRGFFFSHMGWLMCRKSKQVKEKGKEPDISDLYADPILRYQKKYYMLFMPLMCFAFPTVVPLYFWNESLKTAFFVNIFRYIFSLHATWLVNSAAHLYGEKPYNKHINPAENLAVSLIVNGERWHNYHHTFPWDYKAGEFGRYGTNLTTVFINAMAKIGLAYDLKFVPEDVVKRRVHKTGDGSHAVWGWGDKDQTVEEISKTIVAYNQS

SEQ ID NO: 15 - DNA, 909 bp, synthetic construct
  misc_feature 1..909: note = codon-optimized nucleotide sequence
  misc_feature 1..909: note = Y. lipolytica codon-optimized nucleotide sequence of desaturasefrom Tribolium castaneum D6
  source 1..909: mol_type = other DNA
atgttcctgcgaaccatcacctctaagttctactctgaccagatcgtgtggcgaaacgtgttcctgctgctgatcctgcacatcatctccctgcaaggctggtacttcgtgctgaccaccaccaactggcccactctgatctacggcttcatcttcggcgccctgaccggccagggaatcaagctgggagcccaccgactgtgggctcaccgatgctacaaggccaagctgcccctgcgaatcttcctgtgcttcctgcagaccgtgactctgcagaaccctctgtacgagtgggtgcgagatcaccaggtgcaccacaagtacaccgacaccaacgctgaccctctgaacgctacccgaggcttcttcttctctcacatgggctggctgctggtgcgaaagcaccccaacgtgatcgccaagggcaagaccctggacctgtctgacctggaagaggaccccgtggtgatgttccagaagaagtactacaagatcattgcccctgtgctgaccctggctatccccgctctgatcccctggtactttttcggcgaggacctgtacctgtcttgggtgaccacctgtgtgctgccctacttcatcaccctgcactctacctgggccgtgaactctgtggcccacatctggggcaccaagccttacaacaagaacattctgcccaccgagaacattgccgtggccattgtggcctacggcgaaggctggcacaactaccaccacgtgttcccttgggactacaaggctgccgagctgggcaactaccgacctaacctgtctaccgccttcatcgacttcatggccaagatcgcctgggcctacgacctgaagtctgtgtctcccgagatgctgcgaaagcgaaagatgcgaaccggcgactgcgactactaa

SEQ ID NO: 16 - protein, 302 aa, Tribolium castaneum
MFLRTITSKFYSDQIVWRNVFLLLILHIISLQGWYFVLTTTNWPTLIYGFIFGALTGQGIKLGAHRLWAHRCYKAKLPLRIFLCFLQTVTLQNPLYEWVRDHQVHHKYTDTNADPLNATRGFFFSHMGWLLVRKHPNVIAKGKTLDLSDLEEDPVVMFQKKYYKIIAPVLTLAIPALIPWYFFGEDLYLSWVTTCVLPYFITLHSTWAVNSVAHIWGTKPYNKNILPTENIAVAIVAYGEGWHNYHHVFPWDYKAAELGNYRPNLSTAFIDFMAKIAWAYDLKSVSPEMLRKRKMRTGDCDY

SEQ ID NO: 17 - DNA, 1170 bp, synthetic construct
  misc_feature 1..1170: note = codon-optimized nucleotide sequence
  misc_feature 1..1170: note = Y. lipolytica codon-optimized nucleotide sequence of desaturasefrom Tribolium castaneum D8
  source 1..1170: mol_type = other DNA
atggctcccaacctgctgggcaactctaccctgttcctggccgagactaactctgctgagcccatccagatcatctctaagcccggcctgcaggacgtgctgccccaggtgaagccccagatctcttctcgatcttctgtgtctcagtaccgatggcagatcgtgtggcgaaacgtgctgatcttcatctacctgcacattgccggcatctacggcctgtactacgccattgctcaggcccagtggaagaccctgctgtggggctacctggtgatcctggcctctggcatcggcgtgaccgctggcgcccaccgactgtgggctcaccgaacctacaaggccaagctgcccctgcgaatctacctggccttctgccagaccgtggctctgcagaacgacatctacgagtgggtgcgagatcaccgagtgcaccacaagttcaccgacaccgacgctgaccctcacaactctaaccgaggcttcttcttctctcacatgggctggctgctggtgaagaagcacaaggacgttttcgtgaagggcaagaccgtggacatgtctgacgtcgaggctgaccccgtggtgcgattccagcgaaagtactacatcattctgacccctatcctgaccttcgtgttccccgctatcgtgccctggtacttctggaacgagactcccaccgtgtgcttctactctgtggccatcttccgatatatcctgactctgcacggcacctggctggtgaactctgccgctcacatctggggataccgaccttacgacaagaacatcaacgccaccgagaacaagtctgtgtctattctggccttcggcgaaggatggcacaactaccaccacgtgttcccttgggactacaaggctgccgagctgggaaactaccgaatgaacttcaccaccgcctttctggacctgatgtctaagatcggccaggcctacgacctcaagactgtgtctgtggacatgatcaacaagcgacgaaagcgaaccggcgacggaaccggcctggtggacgaggaactgctcgagaacgaggacaagcaccaccaccatcacgacgactctatttggggctggggcgacaaggacatgaagcaggacgacatggacatggtccaggtgcacaacccttctcgagagaagttcgactaa

SEQ ID NO: 18 - protein, 389 aa, Tribolium castaneum
MAPNLLGNSTLFLAETNSAEPIQIISKPGLQDVLPQVKPQISSRSSVSQYRWQIVWRNVLIFIYLHIAGIYGLYYAIAQAQWKTLLWGYLVILASGIGVTAGAHRLWAHRTYKAKLPLRIYLAFCQTVALQNDIYEWVRDHRVHHKFTDTDADPHNSNRGFFFSHMGWLLVKKHKDVFVKGKTVDMSDVEADPVVRFQRKYYIILTPILTFVFPAIVPWYFWNETPTVCFYSVAIFRYILTLHGTWLVNSAAHIWGYRPYDKNINATENKSVSILAFGEGWHNYHHVFPWDYKAAELGNYRMNFTTAFLDLMSKIGQAYDLKTVSVDMINKRRKRTGDGTGLVDEELLENEDKHHHHHDDSIWGWGDKDMKQDDMDMVQVHNPSREKFD

SEQ ID NO: 19 - DNA, 1578 bp, Saccharomyces cerevisiae
  source 1..1578: mol_type = genomic DNA
atgaatgaaatcgatgagaaaaatcaggcccccgtgcaacaagaatgcctgaaagagatgattcagaatgggcatgctcggcgtatgggatctgttgaagatctgtatgttgctctcaacagacaaaacttatatcgaaacttctgcacatatggagaattgagtgattactgtactagggatcagctcacattagctttgagggaaatctgcctgaaaaatccaactcttttacatattgttctaccaacaagatggccaaatcatgaaaattattatcgcagttccgaatactattcacggccacatccagtgcatgattatatttcagtattacaagaattgaaactgagtggtgtggttctcaatgaacaacctgagtacagtgcagtaatgaagcaaatattagaagaattcaaaaatagtaagggttcctatactgcaaaaatttttaaacttactaccactttgactattccttactttggaccaacaggaccgagttggcggctaatttgtcttccagaagagcacacagaaaagtggaaaaaatttatctttgtatctaatcattgcatgtctgatggtcggtcttcgatccacttttttcatgatttaagagacgaattaaataatattaaaactccaccaaaaaaattagattacattttcaagtacgaggaggattaccaattattgaggaaacttccagaaccgatcgaaaaggtgatagactttagaccaccgtacttgtttattccgaagtcacttctttcgggtttcatctacaatcatttgagattttcttcaaaaggtgtctgtatgagaatggatgatgtggaaaaaaccgatgatgttgtcaccgagatcatcaatatttcaccaacagaatttcaagcgattaaagcaaatattaaatcaaatatccaaggtaagtgtactatcactccgtttttacatgtttgttggtttgtatctcttcataaatggggtaaatttttcaaaccattgaacttcgaatggcttacggatatttttatccccgcagattgccgctcacaactaccagatgatgatgaaatgagacagatgtacagatatggcgctaacgttggatttattgacttcaccccctggataagcgaatttgacatgaatgataacaaagaaaatttttggccacttattgagcactaccatgaagtaatttcggaagctttaagaaataaaaagcatctccatggcttagggttcaatatacaaggcttcgttcaaaaatatgtgaacattgacaaggtaatgtgcgatcgtgccatcgggaaaagacgcggaggtacattgttaagcaatgtaggtctgtttaatcagttagaggagcccgatgccaaatattctatatgcgatttggcatttggccaatttcaaggatcctggcaccaagcattttccttgggtgtttgttcgactaatgtaaaggggatgaatattgttgttgcttcaacaaagaatgttgttggtagtcaagaatctctcgaagagctttgctccatttacaaagctctccttttaggcccttag

SEQ ID NO: 20 - DNA, 1578 bp, synthetic construct
  misc_feature 1..1578: note = codon-optimized nucleotide sequence
  misc_feature 1..1578: note = Y.lipolytica codon-optimized nucleotide sequence of alcoholacetyltransferase from S. cerevisiae ATF1
  source 1..1578: mol_type = other DNA
atgaacgagatcgacgagaagaaccaggctcctgtgcagcaagagtgcctgaaggaaatgatccagaacggacacgcccgacgaatgggctctgtcgaggacctgtacgtggccctgaaccgacagaacctgtaccgaaacttctgcacctacggcgagctgtctgactactgcacccgagatcagctgaccctggctctgcgagagatctgcctgaagaaccctactctgctgcatatcgtgctgcccactcgatggcccaaccacgagaactactaccgatcttctgagtactactctcgaccccatcctgtgcacgactacatctccgtgctgcaagagctgaagctgtctggcgtggtgctgaacgagcagcccgagtactctgccgtgatgaagcagatcctggaagagttcaagaactctaagggctcttacaccgccaagatcttcaagctgactactaccctgaccattccttacttcggccccactggaccctcttggcgactgatctgtctgcccgaggaacacaccgagaagtggaagaagttcatcttcgtttctaaccactgcatgtctgacggacgatcctctatccacttctttcacgacctgcgagatgagctgaacaacatcaagacccctccaaagaagctggactacattttcaagtacgaagaggactaccagctgctgcgaaagctgcccgagcctatcgagaaggtgatcgacttccgacctccttacctgttcatccccaagtctctgctgtctggattcatctacaaccacctccgattctcttcgaagggcgtgtgcatgcgaatggacgacgtggaaaagaccgacgacgttgtgaccgagatcatcaacatctctcccaccgagttccaggccatcaaggccaacattaagtctaacatccagggcaagtgtaccatcactccctttctgcacgtgtgctggttcgtgtctctgcacaagtggggcaagttctttaagcccctgaacttcgagtggctgaccgacatcttcatccccgccgactgccgatctcagctgcctgacgacgacgagatgcgacagatgtaccgatacggcgccaacgtgggcttcatcgacttcaccccttggatctctgagttcgacatgaacgacaacaaggaaaacttctggcccctgatcgagcactaccacgaggtgatttctgaggccctgcgaaacaagaagcacctccacggcctgggcttcaacattcagggcttcgtccagaagtacgtcaacattgacaaggtgatgtgcgaccgagccatcggcaagcgacgaggcggcaccctgctgtctaacgtgggcctgttcaaccagctcgaggaacccgacgccaagtactctatctgcgacctggccttcggccagttccaaggctcttggcaccaggctttctccctgggcgtgtgttctaccaacgtgaagggcatgaacatcgtggtggcctctaccaagaacgtggtgggctctcaagagtctctggaagaactgtgctctatctacaaggccctgctgctgggcccctaa

SEQ ID NO: 21 - protein, 525 aa, Saccharomyces cerevisiae
MNEIDEKNQAPVQQECLKEMIQNGHARRMGSVEDLYVALNRQNLYRNFCTYGELSDYCTRDQLTLALREICLKNPTLLHIVLPTRWPNHENYYRSSEYYSRPHPVHDYISVLQELKLSGVVLNEQPEYSAVMKQILEEFKNSKGSYTAKIFKLTTTLTIPYFGPTGPSWRLICLPEEHTEKWKKFIFVSNHCMSDGRSSIHFFHDLRDELNNIKTPPKKLDYIFKYEEDYQLLRKLPEPIEKVIDFRPPYLFIPKSLLSGFIYNHLRFSSKGVCMRMDDVEKTDDVVTEIINISPTEFQAIKANIKSNIQGKCTITPFLHVCWFVSLHKWGKFFKPLNFEWLTDIFIPADCRSQLPDDDEMRQMYRYGANVGFIDFTPWISEFDMNDNKENFWPLIEHYHEVISEALRNKKHLHGLGFNIQGFVQKYVNIDKVMCDRAIGKRRGGTLLSNVGLFNQLEEPDAKYSICDLAFGQFQGSWHQAFSLGVCSTNVKGMNIVVASTKNVVGSQESLEELCSIYKALLLGP

SEQ ID NO: 22 - DNA, 1236 bp, synthetic construct
  misc_feature 1..1236: note = codon-optimized nucleotide sequence
  misc_feature 1..1236: note = Y.lipolytica codon-optimized nucleotide sequence of thioesterasefrom Cuphea palustris CpFATB2
  source 1..1236: mol_type = other DNA
atggtggccgctgccgcctccgccgccttcttctctgtggccacccctcgaactaacatctctccctcgtctctgtctgtgcccttcaagcccaagtctaaccacaacggcggcttccaggtgaaggccaacgcctctgcccaccccaaggccaacggatctgccgtgtctctgaagtctggctctctcgagactcaggaggacaagacctcttcttcgtcgcctcctccccgaaccttcatcaaccagctgcccgtgtggtctatgctgctgtctgccgtgaccaccgtgttcggcgtggccgagaagcagtggcccatgctggaccgaaagtctaagcgacccgacatgctggtcgagcccctgggcgtggaccgaatcgtgtacgacggcgtgtctttccgacagtctttctctatccgatcttacgagatcggcgctgaccgaaccgcctctatcgagactctgatgaacatgttccaggagacttctctgaaccactgcaagatcatcggcctgctgaacgacggcttcggccgaacccctgagatgtgcaagcgagatctgatttgggtggtgaccaagatgcagatcgaggtgaaccgataccccacctggggcgacaccattgaggtgaacacctgggtgtctgcctctggcaagcacggcatgggccgagactggctgatctctgactgccacaccggcgagatcctgatccgagccacctctgtgtgggccatgatgaaccagaagacccgacgactgtctaagatcccctacgaggtgcgacaggagatcgagccccagttcgtggactctgctcccgtgatcgtggacgaccgaaagttccacaagctggacctcaagaccggcgactctatctgcaacggcctgacccctcgatggaccgacctggacgtgaaccagcacgtgaacaacgtgaagtacatcggctggatcctgcagtctgtgcccaccgaggtgtttgagactcaggagctgtgcggcctgaccctcgagtaccgacgagagtgcggccgagactctgtgctcgagtctgtgaccgccatggacccctctaaggagggcgaccgatctctgtaccagcacctcctgcgactcgaggacggcgccgacatcgtgaagggccgaaccgagtggcgacccaagaacgctggcgccaagggcgccatcctgaccggcaagacctctaacggcaactctatctcttaa

SEQ ID NO: 23 - protein, 411 aa, Cuphea palustris
MVAAAASAAFFSVATPRTNISPSSLSVPFKPKSNHNGGFQVKANASAHPKANGSAVSLKSGSLETQEDKTSSSSPPPRTFINQLPVWSMLLSAVTTVFGVAEKQWPMLDRKSKRPDMLVEPLGVDRIVYDGVSFRQSFSIRSYEIGADRTASIETLMNMFQETSLNHCKIIGLLNDGFGRTPEMCKRDLIWVVTKMQIEVNRYPTWGDTIEVNTWVSASGKHGMGRDWLISDCHTGEILIRATSVWAMMNQKTRRLSKIPYEVRQEIEPQFVDSAPVIVDDRKFHKLDLKTGDSICNGLTPRWTDLDVNQHVNNVKYIGWILQSVPTEVFETQELCGLTLEYRRECGRDSVLESVTAMDPSKEGDRSLYQHLLRLEDGADIVKGRTEWRPKNAGAKGAILTGKTSNGNSIS

SEQ ID NO: 24 - DNA, 1368 bp, synthetic construct
  misc_feature 1..1368: note = codon-optimized nucleotide sequence
  misc_feature 1..1368: note = S. cerevisiae-codon-optimized nucleotide sequence of Helicoverpaarmigera fatty acyl reductase; mRNA-coding sequence
  source 1..1368: mol_type = other DNA
atggttgtcttgacctccaaagaaactaagccatctgttgctgaattttacgctggtaagtctgttttcattactggtggtactggtttcttgggtaaggttttcattgaaaagttgttgtactcctgcccagatatcggtaatatctacatgttgatcagagaaaagaagggtttgtccgtttccgaaagaatcaagcactttttggatgatcctttgttcaccagattgaaagaaaaaagaccagccgacttggaaaagatcgttttgattccaggtgatattactgctccagatttgggtattacctccgaaaacgaaaagatgttgatcgaaaaggtcagtgtcattattcattctgctgctaccgttaagttcaacgaaccattgccaactgcttggaagattaacgttgaaggtactagaatgatgttggccttgtctagaagaatgaagagaatcgaagttttcatccatatctctaccgcttacactaacaccaacagagaagttgttgacgaaatcttgtatccagctccagctgatattgatcaagttcacagatatgttaaggacggtatctctgaagaagaaactgaaaaaatcttgaacggtagaccaaacacttacactttcactaaggctttgaccgaacatttggttgctgaaaatcaagcttacgttccaaccattatcgttagaccatcagttgttgctgccattaaggatgaacctattaagggttggttgggtaattggtatggtgctacaggtttgactgtttttactgctaagggtttgaacagagttatctacggtcactcttctaacatcgttgatttgatcccagttgattacgttgccaacttggttattgctgctggtgctaaatcttctaagtctactgaattgaaggtctacaactgctgttcttctgcttgtaacccaattactatcggtaagttgatgtccatgtttgctgaagatgctatcaagcaaaagtcttacgctatgccattgccaggttggtacatttttactaagtacaagtggttggtcttgttgttgaccattttgttccaagttattccagcctacattaccgacttgtacagacatttgattggtaagaacccaagatatatcaagttgcaatccttggtcaatcaaaccagatcctccattgatttcttcacctctcattcttgggttatgaaggctgatagagtcagagaattattcgcttctttgtctccagcagataagtacttgtttccatgtgatccaaccgatattaactggacccattacattcaagattactgctggggtgttagacatttcttggaaaaaaaaagctacgaataa

SEQ ID NO: 25 - protein, 455 aa, Helicoverpa armigera
MVVLTSKETKPSVAEFYAGKSVFITGGTGFLGKVFIEKLLYSCPDIGNIYMLIREKKGLSVSERIKHFLDDPLFTRLKEKRPADLEKIVLIPGDITAPDLGITSENEKMLIEKVSVIIHSAATVKFNEPLPTAWKINVEGTRMMLALSRRMKRIEVFIHISTAYTNTNREVVDEILYPAPADIDQVHRYVKDGISEEETEKILNGRPNTYTFTKALTEHLVAENQAYVPTIIVRPSVVAAIKDEPIKGWLGNWYGATGLTVFTAKGLNRVIYGHSSNIVDLIPVDYVANLVIAAGAKSSKSTELKVYNCCSSACNPITIGKLMSMFAEDAIKQKSYAMPLPGWYIFTKYKWLVLLLTILFQVIPAYITDLYRHLIGKNPRYIKLQSLVNQTRSSIDFFTSHSWVMKADRVRELFASLSPADKYLFPCDPTDINWTHYIQDYCWGVRHFLEKKSYE

SEQ ID NO: 26 - DNA, 1365 bp, synthetic construct
  misc_feature 1..1365: note = codon-optimized nucleotide sequence
  misc_feature 1..1365: note = S. cerevisiae-codon-optimized nucleotide sequence of H. armigerafatty acyl reductase with signal peptide changed to HDEL; DNAcoding sequence.
  source 1..1365: mol_type = other DNA
atggttgtcttgacctccaaagaaactaagccatctgttgctgaattttacgctggtaagtctgttttcattactggtggtactggtttcttgggtaaggttttcattgaaaagttgttgtactcctgcccagatatcggtaatatctacatgttgatcagagaaaagaagggtttgtccgtttccgaaagaatcaagcactttttggatgatcctttgttcaccagattgaaagaaaaaagaccagccgacttggaaaagatcgttttgattccaggtgatattactgctccagatttgggtattacctccgaaaacgaaaagatgttgatcgaaaaggtcagtgtcattattcattctgctgctaccgttaagttcaacgaaccattgccaactgcttggaagattaacgttgaaggtactagaatgatgttggccttgtctagaagaatgaagagaatcgaagttttcatccatatctctaccgcttacactaacaccaacagagaagttgttgacgaaatcttgtatccagctccagctgatattgatcaagttcacagatatgttaaggacggtatctctgaagaagaaactgaaaaaatcttgaacggtagaccaaacacttacactttcactaaggctttgaccgaacatttggttgctgaaaatcaagcttacgttccaaccattatcgttagaccatcagttgttgctgccattaaggatgaacctattaagggttggttgggtaattggtatggtgctacaggtttgactgtttttactgctaagggtttgaacagagttatctacggtcactcttctaacatcgttgatttgatcccagttgattacgttgccaacttggttattgctgctggtgctaaatcttctaagtctactgaattgaaggtctacaactgctgttcttctgcttgtaacccaattactatcggtaagttgatgtccatgtttgctgaagatgctatcaagcaaaagtcttacgctatgccattgccaggttggtacatttttactaagtacaagtggttggtcttgttgttgaccattttgttccaagttattccagcctacattaccgacttgtacagacatttgattggtaagaacccaagatatatcaagttgcaatccttggtcaatcaaaccagatcctccattgatttcttcacctctcattcttgggttatgaaggctgatagagtcagagaattattcgcttctttgtctccagcagataagtacttgtttccatgtgatccaaccgatattaactggacccattacattcaagattactgctggggtgttagacatttcttggaacatgatgaattgtaa

SEQ ID NO: 27 - protein, 454 aa, Helicoverpa armigera
  REGION 1..454: note = MISC_FEATURE - H. armigera fatty acyl reductase with signal peptide changed toHDEL
MVVLTSKETKPSVAEFYAGKSVFITGGTGFLGKVFIEKLLYSCPDIGNIYMLIREKKGLSVSERIKHFLDDPLFTRLKEKRPADLEKIVLIPGDITAPDLGITSENEKMLIEKVSVIIHSAATVKFNEPLPTAWKINVEGTRMMLALSRRMKRIEVFIHISTAYTNTNREVVDEILYPAPADIDQVHRYVKDGISEEETEKILNGRPNTYTFTKALTEHLVAENQAYVPTIIVRPSVVAAIKDEPIKGWLGNWYGATGLTVFTAKGLNRVIYGHSSNIVDLIPVDYVANLVIAAGAKSSKSTELKVYNCCSSACNPITIGKLMSMFAEDAIKQKSYAMPLPGWYIFTKYKWLVLLLTILFQVIPAYITDLYRHLIGKNPRYIKLQSLVNQTRSSIDFFTSHSWVMKADRVRELFASLSPADKYLFPCDPTDINWTHYIQDYCWGVRHFLEHDEL

SEQ ID NO: 28 - DNA, 1371 bp, synthetic construct
  misc_feature 1..1371: note = codon-optimized nucleotide sequence
  misc_feature 1..1371: note = S. cerevisiae-codon-optimized nucleotide sequence of H. assultafatty acyl reductase; mRNA-coding sequence
  source 1..1371: mol_type = other DNA
atggttgtcttgacctccaaagaaactaagccatctgttgctgaattttacgctggtaagtctgttttcattactggtggtactggtttcttgggtaagatcttcattgaaaagttgttgtactcctgcccagatatcggtaatatctacatgttgatcagagaaaagaagggtttgtccgtttccgaaagaatcaagcaatttttggatgaccctttgttcaccagattgaaagaaaaaagaccagccgacttggaaaagatcgttttgattccaggtgatattactgctccagatttgggtattacctccgaaaacgaaaagatgttgatcgaaaaggtcagtgtcattattcattctgctgctaccgttaagttcaacgaaccattgccaactgcttggaagattaacgttgaaggtactagaatgatgttggccttgtctagaagaatgaagagaatcgaagttttcatccatatctctaccgcttacactaacaccaacagagaagttgttgacgaaatcttgtatccagctccagctgatattgatcaagttcaccaatatgttaaggacggtatctctgaagaagaaactgaaaaaatcttgaacggtagaccaaacacttacactttcactaaggctttgaccgaacatttggttgctgaaaatcaagcttacgttccaaccattatcgttagaccatcagttgttgctgccattaaggatgaacctattaagggttggttgggtaattggtatggtgctacaggtttgactgtttttactgctaagggtttgaacagagttatctacggtcattcctcttacatcgttgatttgatcccagttgattacgttgccaacttggttattgctgctggtgctaaatcttctaagtctactgaattgaaggtctacaactgctgttcttctgcttgtaacccaattactatcggtaagttgatgtccatgtttgctgaagatgctatcaagcaaaagtcttacgctatgccattgccaggttggtatgtttttacaaagtacaagtggttggtcttgttgttgaccattttgttccaagttattccagcctacattaccgacttgtacagacatttgattggtaagaacccaagatatatcaagttgcaatccttggtcaatcaaaccagatcctccattgatttcttcacctctcattcttgggttatgaaggctgatagagtcagagaattattcgcttctttgtctccagcagataagtacttgtttccatgtgatccaaccgatattaactggacccattacattcaagattactgctggggtgttagacacttcttggaaaaaaagactaccaacaagtaa

SEQ ID NO: 29 - protein, 456 aa, Helicoverpa assulta
MVVLTSKETKPSVAEFYAGKSVFITGGTGFLGKIFIEKLLYSCPDIGNIYMLIREKKGLSVSERIKQFLDDPLFTRLKEKRPADLEKIVLIPGDITAPDLGITSENEKMLIEKVSVIIHSAATVKFNEPLPTAWKINVEGTRMMLALSRRMKRIEVFIHISTAYTNTNREVVDEILYPAPADIDQVHQYVKDGISEEETEKILNGRPNTYTFTKALTEHLVAENQAYVPTIIVRPSVVAAIKDEPIKGWLGNWYGATGLTVFTAKGLNRVIYGHSSYIVDLIPVDYVANLVIAAGAKSSKSTELKVYNCCSSACNPITIGKLMSMFAEDAIKQKSYAMPLPGWYVFTKYKWLVLLLTILFQVIPAYITDLYRHLIGKNPRYIKLQSLVNQTRSSIDFFTSHSWVMKADRVRELFASLSPADKYLFPCDPTDINWTHYIQDYCWGVRHFLEKKTTNK

SEQ ID NO: 30 - DNA, 1365 bp, synthetic construct
  misc_feature 1..1365: note = codon-optimized nucleotide sequence
  misc_feature 1..1365: note = S. cerevisiae-codon-optimized nucleotide sequence of Helicoverpaassulta fatty acyl reductase with signal peptide changed to HDEL;mRNA-coding sequence
  source 1..1365: mol_type = other DNA
atggttgtcttgacctccaaagaaactaagccatctgttgctgaattttacgctggtaagtctgttttcattactggtggtactggtttcttgggtaagatcttcattgaaaagttgttgtactcctgcccagatatcggtaatatctacatgttgatcagagaaaagaagggtttgtccgtttccgaaagaatcaagcaatttttggatgaccctttgttcaccagattgaaagaaaaaagaccagccgacttggaaaagatcgttttgattccaggtgatattactgctccagatttgggtattacctccgaaaacgaaaagatgttgatcgaaaaggtcagtgtcattattcattctgctgctaccgttaagttcaacgaaccattgccaactgcttggaagattaacgttgaaggtactagaatgatgttggccttgtctagaagaatgaagagaatcgaagttttcatccatatctctaccgcttacactaacaccaacagagaagttgttgacgaaatcttgtatccagctccagctgatattgatcaagttcaccaatatgttaaggacggtatctctgaagaagaaactgaaaaaatcttgaacggtagaccaaacacttacactttcactaaggctttgaccgaacatttggttgctgaaaatcaagcttacgttccaaccattatcgttagaccatcagttgttgctgccattaaggatgaacctattaagggttggttgggtaattggtatggtgctacaggtttgactgtttttactgctaagggtttgaacagagttatctacggtcattcctcttacatcgttgatttgatcccagttgattacgttgccaacttggttattgctgctggtgctaaatcttctaagtctactgaattgaaggtctacaactgctgttcttctgcttgtaacccaattactatcggtaagttgatgtccatgtttgctgaagatgctatcaagcaaaagtcttacgctatgccattgccaggttggtatgtttttacaaagtacaagtggttggtcttgttgttgaccattttgttccaagttattccagcctacattaccgacttgtacagacatttgattggtaagaacccaagatatatcaagttgcaatccttggtcaatcaaaccagatcctccattgatttcttcacctctcattcttgggttatgaaggctgatagagtcagagaattattcgcttctttgtctccagcagataagtacttgtttccatgtgatccaaccgatattaactggacccattacattcaagattactgctggggtgttagacacttcttggaacatgatgaattgtaa

SEQ ID NO: 31 - protein, 454 aa, Helicoverpa assulta
  REGION 1..454: note = MISC_FEATURE - amino acid sequence of H. assulta fatty acyl reductase withsignal peptide changed to HDEL
MVVLTSKETKPSVAEFYAGKSVFITGGTGFLGKIFIEKLLYSCPDIGNIYMLIREKKGLSVSERIKQFLDDPLFTRLKEKRPADLEKIVLIPGDITAPDLGITSENEKMLIEKVSVIIHSAATVKFNEPLPTAWKINVEGTRMMLALSRRMKRIEVFIHISTAYTNTNREVVDEILYPAPADIDQVHQYVKDGISEEETEKILNGRPNTYTFTKALTEHLVAENQAYVPTIIVRPSVVAAIKDEPIKGWLGNWYGATGLTVFTAKGLNRVIYGHSSYIVDLIPVDYVANLVIAAGAKSSKSTELKVYNCCSSACNPITIGKLMSMFAEDAIKQKSYAMPLPGWYVFTKYKWLVLLLTILFQVIPAYITDLYRHLIGKNPRYIKLQSLVNQTRSSIDFFTSHSWVMKADRVRELFASLSPADKYLFPCDPTDINWTHYIQDYCWGVRHFLEHDEL

SEQ ID NO: 32 - DNA, 1362 bp, synthetic construct
  misc_feature 1..1362: note = codon-optimized nucleotide sequence
  misc_feature 1..1362: note = S. cerevisiae-codon-optimized nucleotide sequence of Heliothissubflexa fatty acyl reductase; mRNA-coding sequence.
  source 1..1362: mol_type = other DNA
atggttgtcttgacctccaaagaaactaagccatctgttgctgaattttacgctggtaagtctgttttcattactggtggtactggtttcttgggtaaggttttcattgaaaagttgttgtactcctgcccagatatcggtaatatctacatgttgatcagagaaaagaagggtttgtccgtttccgaaagaatcaagcactttttggatgatcctttgttcaccagattgaaagaaaaaagaccagccgacttggaaaagatcgttttgattccaggtgatattactgctccagatttgggtattacctccgaaaacgaaaagatgttgatcgaaaaggtcagtgtcattattcattctgctgctaccgttaagttcaacgaaccattgccaactgcttggaagattaacgttgaaggtactagaatgatgttggccttgtctagaagaatgaagagaatcgaagttttcatccatatctctaccgcttacactaacaccaacagagaagttgttgacgaaatcttgtatccagctccagctgatattgatcaagttcaccaatatgttaaggacggtatctctgaagaagaaactgaaaaaatcttgaacggtagaccaaacacttacactttcactaaggctttgaccgaacatttggttgctgaaaatcaagcttacgttccaaccattatcgttagaccatcagttgttgctgccattaaggatgaacctattaagggttggttgggtaattggtatggtgctacaggtttgactgtttttactgctaagggtttgaacagagttatctacggtcactcttctaacatcgttgatttgatcccagttgattacgttgccaacttggttattgctgctggtgctaaatcttctaagtctactgaattgaaggtctacaactgctgttcttctgcttgtaacccaattactatcggtaagttgatgtccatgtttgctgaagatgctatcaagcaaaagtcttacgctatgccattgccaggttggtacatttttactaagtacaagtggttggtcttgttgttgaccattttgttccaagttattccagcctacattaccgacttgtacagacatttgattggtaagaacccaagatatatcaagttgcaatccttggtcaatcaaaccagatcctccattgatttcttcaccaaccattcttgggttatgaaggctgatagagtcagagaattattcgcttctttgtctccagcagataagtacttgtttccatgtgatccagtcaacatcaattggagacaatatatccaagattactgctggggtgttagacatttcttggaaaaaaagacttaa

SEQ ID NO: 33 - protein, 453 aa, Heliothis subflexa
MVVLTSKETKPSVAEFYAGKSVFITGGTGFLGKVFIEKLLYSCPDIGNIYMLIREKKGLSVSERIKHFLDDPLFTRLKEKRPADLEKIVLIPGDITAPDLGITSENEKMLIEKVSVIIHSAATVKFNEPLPTAWKINVEGTRMMLALSRRMKRIEVFIHISTAYTNTNREVVDEILYPAPADIDQVHQYVKDGISEEETEKILNGRPNTYTFTKALTEHLVAENQAYVPTIIVRPSVVAAIKDEPIKGWLGNWYGATGLTVFTAKGLNRVIYGHSSNIVDLIPVDYVANLVIAAGAKSSKSTELKVYNCCSSACNPITIGKLMSMFAEDAIKQKSYAMPLPGWYIFTKYKWLVLLLTILFQVIPAYITDLYRHLIGKNPRYIKLQSLVNQTRSSIDFFTNHSWVMKADRVRELFASLSPADKYLFPCDPVNINWRQYIQDYCWGVRHFLEKKT

SEQ ID NO: 34 - DNA, 1362 bp, synthetic construct
  misc_feature 1..1362: note = codon-optimized nucleotide sequence
  misc_feature 1..1362: note = S. cerevisiae-codon-optimized nucleotide sequence of H. subflexafatty acyl reductase with signal peptide changed to HDEL;mRNA-coding sequence
  source 1..1362: mol_type = other DNA
atggttgtcttgacctccaaagaaactaagccatctgttgctgaattttacgctggtaagtctgttttcattactggtggtactggtttcttgggtaaggttttcattgaaaagttgttgtactcctgcccagatatcggtaatatctacatgttgatcagagaaaagaagggtttgtccgtttccgaaagaatcaagcactttttggatgatcctttgttcaccagattgaaagaaaaaagaccagccgacttggaaaagatcgttttgattccaggtgatattactgctccagatttgggtattacctccgaaaacgaaaagatgttgatcgaaaaggtcagtgtcattattcattctgctgctaccgttaagttcaacgaaccattgccaactgcttggaagattaacgttgaaggtactagaatgatgttggccttgtctagaagaatgaagagaatcgaagttttcatccatatctctaccgcttacactaacaccaacagagaagttgttgacgaaatcttgtatccagctccagctgatattgatcaagttcaccaatatgttaaggacggtatctctgaagaagaaactgaaaaaatcttgaacggtagaccaaacacttacactttcactaaggctttgaccgaacatttggttgctgaaaatcaagcttacgttccaaccattatcgttagaccatcagttgttgctgccattaaggatgaacctattaagggttggttgggtaattggtatggtgctacaggtttgactgtttttactgctaagggtttgaacagagttatctacggtcactcttctaacatcgttgatttgatcccagttgattacgttgccaacttggttattgctgctggtgctaaatcttctaagtctactgaattgaaggtctacaactgctgttcttctgcttgtaacccaattactatcggtaagttgatgtccatgtttgctgaagatgctatcaagcaaaagtcttacgctatgccattgccaggttggtacatttttactaagtacaagtggttggtcttgttgttgaccattttgttccaagttattccagcctacattaccgacttgtacagacatttgattggtaagaacccaagatatatcaagttgcaatccttggtcaatcaaaccagatcctccattgatttcttcaccaaccattcttgggttatgaaggctgatagagtcagagaattattcgcttctttgtctccagcagataagtacttgtttccatgtgatccagtcaacatcaattggagacaatatatccaagattactgctggggtgttagacatttcttgcatgatgaattgtaa

SEQ ID NO: 35 - protein, 453 aa, Heliothis subflexa
  REGION 1..453: note = MISC_FEATURE - amino acid sequence of H. subflexa fatty acyl reductase withsignal peptide changed to HDEL
MVVLTSKETKPSVAEFYAGKSVFITGGTGFLGKVFIEKLLYSCPDIGNIYMLIREKKGLSVSERIKHFLDDPLFTRLKEKRPADLEKIVLIPGDITAPDLGITSENEKMLIEKVSVIIHSAATVKFNEPLPTAWKINVEGTRMMLALSRRMKRIEVFIHISTAYTNTNREVVDEILYPAPADIDQVHQYVKDGISEEETEKILNGRPNTYTFTKALTEHLVAENQAYVPTIIVRPSVVAAIKDEPIKGWLGNWYGATGLTVFTAKGLNRVIYGHSSNIVDLIPVDYVANLVIAAGAKSSKSTELKVYNCCSSACNPITIGKLMSMFAEDAIKQKSYAMPLPGWYIFTKYKWLVLLLTILFQVIPAYITDLYRHLIGKNPRYIKLQSLVNQTRSSIDFFTNHSWVMKADRVRELFASLSPADKYLFPCDPVNINWRQYIQDYCWGVRHFLHDEL

SEQ ID NO: 36 - DNA, 1086 bp, synthetic construct
  misc_feature 1..1086: note = codon-optimized nucleotide sequence
  misc_feature 1..1086: note = Y. lipolytica codon-optimized nucleotide sequence of delta9desaturase from Drosophila melanogaster Dmd9
  source 1..1086: mol_type = other DNA
atggctccctactctcgaatctaccaccaggacaagtcgtcccgagagactggcgtgctgttcgaggacgacgcccagaccgtggactctgacctgaccaccgaccgattccagctgaagcgagccgagaagcgacgactgcccctggtgtggcgaaacatcatcctgttcgccctggtgcacctggccgctctgtacggcctgcactctatcttcacccgagccaagctggccaccactctgttcgctgccggcctgtacatcatcggcatgctgggcgtgaccgctggcgcccaccgactgtgggctcaccgaacctacaaggccaagtggcccctgcgactgctgctggtgatcttcaacaccattgccttccaggacgccgtgtaccactgggcccgagatcaccgagtgcaccacaagtactctgagactgacgctgaccctcacaacgctacccgaggcttcttcttctctcacgtcggctggctgctgtgcaagaagcaccccgacatcaaggaaaagggccgaggcctggacctgtctgacctgcgagctgaccccatcctgatgttccagcgaaagcactactacattctgatgcccctggcctgcttcgtgctgcccaccgtgattcccatggtgtactggaacgagactctggcctcttcctggttcgtggccaccatgttccgatggtgcttccagctcaacatgacctggctggtgaactctgccgctcacaagttcggcaaccgaccttacgacaagactatgaaccccactcagaacgccttcgtgtctgccttcaccttcggcgaaggctggcacaactaccaccacgcattcccttgggactacaagaccgccgagtggggctgctactctctgaacatcaccaccgccttcatcgacctgttcgctaagatcggctgggcctacgacctcaagaccgtggctcccgacgtgatccagcgacgagtgctgcgaaccggcgacggctctcacgagctgtggggctggggcgacaaggacctgaccgctgaggacgcccgaaacgtcctgctggtggacaagtctcgataa

SEQ ID NO: 37 - DNA, 1185 bp, synthetic construct
  misc_feature 1..1185: note = codon-optimized nucleotide sequence
  misc_feature 1..1185: note = Y. lipolytica codon-optimised nucleotide sequence of thioesterasefrom Cuphea hookeriana ChFatB3
  source 1..1185: mol_type = other DNA
atggtggccgctgccgcctcttctgccttcttctcggtgcccactcctggcatctctcccaagcctggcaagttcggcaacggcggcttccaggtgaaggccaacgccaacgctcacccctcgctgaagtctggctctctcgagactgaggacgacacctcttcctcttctccaccacctcgaaccttcatcaaccagctgcctgactggtctatgctgctgtctgccatcaccaccatcttcggagccgccgagaagcagtggatgatgctggaccgaaagtctaagcgacccgacatgctgatggaacccttcggcgtggactctatcgtgcaggacggcgtgttcttccgacagtctttctctatccgatcttacgagattggcgccgaccgaaccacctctatcgagactctgatgaacatgtttcaagagacttctctgaaccactgcaagtctaacggcctgctgaacgacggcttcggacgaacccctgagatgtgcaagaagggcctgatctgggtcgtgaccaagatgcaggtcgaggtgaacagataccccatctggggcgactctattgaggtcaacacctgggtgtctgagtctggcaagaacggcatgggccgagactggctgatctctgactgctctaccggcgagatcctggtgcgagccacctctgtgtgggccatgatgaaccagaagacccgacgactgtctaagttcccattcgaggtgcgacaagagatcgctcccaacttcgtcgactctgtccccgtgatcgaggacgaccgaaagctgcacaagctggacgtcaagaccggcgactccatccacaacggactgacccctcgatggaacgacctggacgtgaaccagcacgtgaacaacgtgaagtacatcggctggatcctgaagtcggtgcccaccgacgtgttcgaggcccaagagctgtgcggcgtgaccctcgagtaccgacgagagtgcggacgagactccgtgatggaatctgtgaccgctatggacccctctaaagaaggcgaccgatctgtctaccagcacctcctgcgactcgaggacggcgccgacattgccatcggccgaaccgagtggcgacccaagaacgctggcgccaacggcgccatctctaccggaaagacctctaaccgaaactctgtgtcttaa

SEQ ID NO: 38 - protein, 394 aa, Cuphea hookeriana
MVAAAASSAFFSVPTPGISPKPGKFGNGGFQVKANANAHPSLKSGSLETEDDTSSSSPPPRTFINQLPDWSMLLSAITTIFGAAEKQWMMLDRKSKRPDMLMEPFGVDSIVQDGVFFRQSFSIRSYEIGADRTTSIETLMNMFQETSLNHCKSNGLLNDGFGRTPEMCKKGLIWVVTKMQVEVNRYPIWGDSIEVNTWVSESGKNGMGRDWLISDCSTGEILVRATSVWAMMNQKTRRLSKFPFEVRQEIAPNFVDSVPVIEDDRKLHKLDVKTGDSIHNGLTPRWNDLDVNQHVNNVKYIGWILKSVPTDVFEAQELCGVTLEYRRECGRDSVMESVTAMDPSKEGDRSVYQHLLRLEDGADIAIGRTEWRPKNAGANGAISTGKTSNRNSVS

SEQ ID NO: 39 - DNA, 1149 bp, synthetic construct
  misc_feature 1..1149: note = codon-optimized nucleotide sequence
  misc_feature 1..1149: note = Y. lipolytica codon-optimised nucleotide sequence of thioesterasefrom Cinnamomum camphora CcFatB1
  source 1..1149: mol_type = other DNA
atggctaccacctctctggcctctgccttctgctctatgaaggccgtgatgctggcccgagatggccgaggaatgaagccccgatcttctgacctgcagctgcgagccggcaacgcccagacctctctgaagatgatcaacggcaccaagttctcttacaccgagtcgctgaagaagctgcccgactggtctatgctgttcgccgtgatcaccaccatcttctctgccgccgagaagcagtggaccaacctcgagtggaagcccaagcctaaccctcctcagctgctggacgaccacttcggaccccacggcctggtgttccgacgaaccttcgccatccgatcttacgaggtgggccccgaccgatctacctctatcgtggccgtcatgaaccacctccaagaggccgctctgaaccacgccaagtctgtgggcatcctcggcgacggcttcggcaccactctcgagatgtctaagcgagatctgatttgggtcgtgaagcgaacccacgtcgccgtcgagcgataccccgcctggggcgacaccgtcgaggtcgagtgctgggtgggcgcctctggcaacaacggccgacgacacgactttctggtgcgagactgcaagaccggcgagattctgacccgatgtacctctctgtctgtgatgatgaacacccgaactcgacgactgtctaagatccccgaggaagtgcgaggcgagatcggacccgccttcatcgacaacgtggccgtgaaggacgaggaaatcaagaagccccagaagctgaacgactctaccgccgactacatccaaggcggactgacccctcgatggaacgacctggacatcaaccagcacgtgaacaacatcaagtacgtggactggatcctcgagactgtgcccgactctatcttcgagtctcaccacatctcttcgttcaccatcgagtaccgacgagagtgcaccatggactctgtgctgcagtctctgaccaccgtgtctggcggctcctctgaggccggactggtgtgcgagcacctcctgcagctcgaaggcggctctgaggtcctgcgagccaagaccgagtggcgacccaagctgactgactctttccgaggcatctctgtgatccccgccgagtcctctgtgtaa

SEQ ID NO: 40 - protein, 382 aa, Cinnamomum camphora
MATTSLASAFCSMKAVMLARDGRGMKPRSSDLQLRAGNAQTSLKMINGTKFSYTESLKKLPDWSMLFAVITTIFSAAEKQWTNLEWKPKPNPPQLLDDHFGPHGLVFRRTFAIRSYEVGPDRSTSIVAVMNHLQEAALNHAKSVGILGDGFGTTLEMSKRDLIWVVKRTHVAVERYPAWGDTVEVECWVGASGNNGRRHDFLVRDCKTGEILTRCTSLSVMMNTRTRRLSKIPEEVRGEIGPAFIDNVAVKDEEIKKPQKLNDSTADYIQGGLTPRWNDLDINQHVNNIKYVDWILETVPDSIFESHHISSFTIEYRRECTMDSVLQSLTTVSGGSSEAGLVCEHLLQLEGGSEVLRAKTEWRPKLTDSFRGISVIPAESSV

SEQ ID NO: 41 - DNA, 627 bp, synthetic construct
  misc_feature 1..627: note = codon-optimized nucleotide sequence
  misc_feature 1..627: note = Y.lipolytica codon-optimized nucleotide sequence of thioesterasefrom Escherichia coli TesA, without the leader sequence, namedTesA(LL)
  source 1..627: mol_type = other DNA
atgatgaacttcaacaacgtgttccgatggcatctgccctttctgtttctggtgctgctgaccttccgagccgccgctgctgacaccctgctgatcctgggcgactctctgtctgccggctaccgaatgtctgcctctgccgcttggcccgctctgctgaacgacaagtggcagtctaagacctctgtggtgaacgcctctatctctggcgacacctctcagcagggcctcgctcgactgcctgctctgctcaagcagcatcagccccgatgggtgctcgtcgagcttggcggcaacgacggcctgcgaggcttccagcctcagcagaccgagcagaccctgcgacagattctgcaggacgtgaaggccgccaacgctgagcctctgctgatgcagattcgactgcccgccaactacggccgacgatacaacgaggccttctctgctatctaccccaagctggccaaggaattcgacgtgcccctgctgccattcttcatggaagaggtgtacctgaagcctcagtggatgcaggacgacggcattcaccccaaccgagatgctcagcccttcattgccgactggatggccaagcagctgcagcctctggtgaaccacgactcttaa

SEQ ID NO: 42 - protein, 208 aa, Escherichia coli
  REGION 1..208: note = MISC_FEATURE - protein sequence of thioesterase from Escherichia coli TesA,without the leader sequence, named TesA(LL)
MMNFNNVFRWHLPFLFLVLLTFRAAAADTLLILGDSLSAGYRMSASAAWPALLNDKWQSKTSVVNASISGDTSQQGLARLPALLKQHQPRWVLVELGGNDGLRGFQPQQTEQTLRQILQDVKAANAEPLLMQIRLPANYGRRYNEAFSAIYPKLAKEFDVPLLPFFMEEVYLKPQWMQDDGIHPNRDAQPFIADWMAKQLQPLVNHDS

SEQ ID NO: 43 - DNA, 1368 bp, synthetic construct
  misc_feature 1..1368: note = codon-optimized nucleotide sequence
  misc_feature 1..1368: note = Y.lipolytica codon-optimized nucleotide sequence of fatty acylreductase from H. armigera Har_FAR
  source 1..1368: mol_type = other DNA
atggtggtcctgacctctaaggagactaagccctccgtggccgagttctacgctggcaagtctgtcttcatcaccggcggaaccggtttcctgggcaaggtcttcattgagaagctgctgtactcctgtcccgacatcggcaacatctacatgctgatccgagagaagaagggactgtctgtgtccgagcgaattaagcacttcctggacgaccccctgttcacccgactgaaggagaagcgacccgccgacctggagaagatcgtgctgattcccggagacatcaccgctcccgacctgggtattacctctgagaacgagaagatgctgatcgagaaggtgtctgtcatcattcactccgccgctaccgtcaagttcaacgagcccctgcccaccgcctggaagatcaacgtggagggaacccgaatgatgctggctctgtctcgacgaatgaagcgaattgaggtcttcatccacatttccaccgcctacaccaacaccaaccgagaggtggtggacgagatcctgtaccctgctcctgctgacattgaccaggtgcaccgatacgtcaaggacggtatctctgaggaagagactgagaagattctgaacggccgacccaacacctacaccttcaccaaggccctgaccgagcacctggtggctgagaaccaggcttacgtgcccaccatcattgtccgaccctccgtggtcgccgctatcaaggacgagcccattaagggatggctgggtaactggtacggagctaccggactgaccgtgttcaccgctaagggtctgaaccgagtcatctacggccactcttccaacatcgtggacctgattcccgtggactacgtcgccaacctggtcattgccgctggcgctaagtcttccaagtccaccgagctgaaggtgtacaactgttgctcttccgcctgcaaccccatcaccattggaaagctgatgtctatgttcgccgaggacgctatcaagcagaagtcctacgctatgcccctgcccggttggtacatcttcaccaagtacaagtggctggtcctgctgctgaccattctgttccaggtcatccccgcctacattaccgacctgtaccgacacctgatcggcaagaacccccgatacattaagctgcagtctctggtcaaccagacccgatcttccattgacttcttcacctctcactcctgggtcatgaaggctgaccgagtccgagagctgttcgcctctctgtcccccgctgacaagtacctgttcccctgtgaccccaccgacatcaactggacccactacattcaggactactgctggggagtgcgacacttcctggagaagaagtcctacgagtag

SEQ ID NO: 44 - DNA, 1437 bp, synthetic construct
  misc_feature 1..1437: note = codon-optimized nucleotide sequence
  misc_feature 1..1437: note = Y.lipolytica codon-optimized nucleotide sequence of fatty acylreductase from Bicyclus anynana Ban-wFAR2
  source 1..1437: mol_type = other DNA
atgtaccgaaacgtgaacaacaactacaagggccactctgtgtacaccaacggcgctggctctcgagtgaagtctctgctgtcctctgccaccgacaacaccaacgagtaccagtctatcgccgagtgctacaagggacagtccgtgttcatcaccggcggcaccggcttcgtcggcaaggtgctgctcgagaagctgctgtactcttgccccggcatcgacaaggtgtacctgctggtgcgagagactcagggcgccaccgctcaccagcgaatgcagaagctcctggaagaacccgccttctcgcgaatcaaggaagagaaccctcaggccttcgagaaggtgatccccatcgtgggcgacatcacccagcctcagctgggcatcatggccgagaacgaggaactgctgattaaggaagtgtctttcgtctaccacgtggccgccaccaccaagttcaacgagactctggacattgccatgaacgtgaacgtggccggaaccggacgagtgctggacctgtctaagcgaatggaaaacatcaaggccttcgtgtacgtgtctaccgcctactctaacaccgaccgagaggtggtggaagaggtgctgtaccccgctcctgtgtctctgaacgaggtgcacaagctgctgaagatcggcatcaccgacgctcaggtgaaggaactgatcaagggacgacccaacacctacaccttcaccaaggctctggctgagaacctggtggccgacaaccacggacacgtgcccgccatcatcgtgcgaccctctatcgtgtcctcgtctaagaaggaacccatcaccggatggatcgactcttggtacggcgccaccttcctggccaccgtgaccatgaagggcttcaaccgagtgttcgtgtcgtcttacgagtacaacctggacttcatccccgtggactacgtgtccaacctgatcatcgtggccgctgctcgatgcaagtgctctgacaaggtggacgtgtacaactcttctacctccggcgaaaaccctctgaagattggcgccttcttcgacgacatcattgcctactcttgcaagcacaagttctacgacatccctctgcctatggcctacctgactcgataccgatgggtcatgttcctgatcaccctgctgctgcagaccctgcctgcctatatcgccgacctgttcctgctgatcgtgggcaagaagccccgatacgtcaagctggcctctaagatctctgccgctcacgaggtcctggactacttcccctctcgaacctggtctatgtctgcccgacagaccaccgctctgttccagtctctgtctccctcggaccgagatcagtttccttgcgaccccaccgacatcgactggaaggagtacatcgtcacctactgccagggaatccgacagttcctgtgcaagtcttaa

SEQ ID NO: 45 - protein, 478 aa, Bicyclus anynana
MYRNVNNNYKGHSVYTNGAGSRVKSLLSSATDNTNEYQSIAECYKGQSVFITGGTGFVGKVLLEKLLYSCPGIDKVYLLVRETQGATAHQRMQKLLEEPAFSRIKEENPQAFEKVIPIVGDITQPQLGIMAENEELLIKEVSFVYHVAATTKFNETLDIAMNVNVAGTGRVLDLSKRMENIKAFVYVSTAYSNTDREVVEEVLYPAPVSLNEVHKLLKIGITDAQVKELIKGRPNTYTFTKALAENLVADNHGHVPAIIVRPSIVSSSKKEPITGWIDSWYGATFLATVTMKGFNRVFVSSYEYNLDFIPVDYVSNLIIVAAARCKCSDKVDVYNSSTSGENPLKIGAFFDDIIAYSCKHKFYDIPLPMAYLTRYRWVMFLITLLLQTLPAYIADLFLLIVGKKPRYVKLASKISAAHEVLDYFPSRTWSMSARQTTALFQSLSPSDRDQFPCDPTDIDWKEYIVTYCQGIRQFLCKS

SEQ ID NO: 46 - DNA, 29 bp, synthetic construct
  misc_feature 1..29: note = Primer sequence
  misc_feature 1..29: note = PR-1852 (PTDH3_fw)n = uracil
  source 1..29: mol_type = other DNA
cacgcganataaaaaacacgctttttcag

SEQ ID NO: 47 - DNA, 34 bp, synthetic construct
  misc_feature 1..34: note = Primer sequence
  misc_feature 1..34: note = pr-1853 (ptdh3_rv)n = uracil
  source 1..34: mol_type = other DNA
acctgcacntttgtttgtttatgtgtgtttattc

SEQ ID NO: 48 - DNA, 26 bp, synthetic construct
  misc_feature 1..26: note = Primer sequence
  misc_feature 1..26: note = pr-1565 (ptef1)n = uracil
  source 1..26: mol_type = other DNA
atgacaganttgtaattaaaacttag

SEQ ID NO: 49 - DNA, 37 bp, synthetic construct
  misc_feature 1..37: note = Primer sequence
  misc_feature 1..37: note = pr-8332 (har_far_u1_fw)n = uracil
  source 1..37: mol_type = other DNA
agtgcaggnaaaacaatggttgtcttgacctccaaag

SEQ ID NO: 50 - DNA, 43 bp, synthetic construct
  misc_feature 1..43: note = Primer sequence
  misc_feature 1..43: note = pr-10739 (har_far_hdel_u1_rev)n = uracil
  source 1..43: mol_type = other DNA
cgtgcganttacaattcatcatgttccaagaaatgtctaacac

SEQ ID NO: 51 - DNA, 33 bp, synthetic construct
  misc_feature 1..33: note = Primer sequence
  misc_feature 1..33: note = pr-14318 (phd9_u2_fw)n = uracil
  source 1..33: mol_type = other DNA
atctgtcanaaaacaatgggcgtcctgctgaac

SEQ ID NO: 52 - DNA, 21 bp, synthetic construct
  misc_feature 1..21: note = Primer sequence
  misc_feature 1..21: note = PR-14276 (Phd9_U2_rev)n = uracil
  source 1..21: mol_type = other DNA
cacgcganttagacctttcgg

SEQ ID NO: 53 - DNA, 27 bp, synthetic construct
  misc_feature 1..27: note = Primer sequence
  misc_feature 1..27: note = pr-14319 (rcd9_u2_fw)n = uracil
  source 1..27: mol_type = other DNA
atctgtcanaaaacaatggccctgaag

SEQ ID NO: 54 - DNA, 23 bp, synthetic construct
  misc_feature 1..23: note = Primer sequence
  misc_feature 1..23: note = pr-14278 (rcd9_u2_rev)
  misc_feature 1..23: note = pr-14278 (rcd9_u2_rev)n = uracil
  source 1..23: mol_type = other DNA
cacgcganttacagcttcacctg

SEQ ID NO: 55 - DNA, 33 bp, synthetic construct
  misc_feature 1..33: note = Primer sequence
  misc_feature 1..33: note = pr-14320 (atf1_u2_fw)n = uracil
  source 1..33: mol_type = other DNA
atctgtcanaaaacaatgaatgaaatcgatgag

SEQ ID NO: 56 - DNA, 33 bp, synthetic construct
  misc_feature 1..33: note = Primer sequence
  misc_feature 1..33: note = pr-14321 (atf1_u2_rev)n = uracil
  source 1..33: mol_type = other DNA
cacgcganctaagggcctaaaaggagagctttg

SEQ ID NO: 57 - DNA, 36 bp, synthetic construct
  misc_feature 1..36: note = Primer sequence
  misc_feature 1..36: note = pr-15974 (dmd9_u1_fw)n = uracil
  source 1..36: mol_type = other DNA
agtgcaggnaaaacaatggctccatactctagaatc

SEQ ID NO: 58 - DNA, 27 bp, synthetic construct
  misc_feature 1..27: note = Primer sequence
  misc_feature 1..27: note = pr-15975 (dmd9_u1_rev)n = uracil
  source 1..27: mol_type = other DNA
cgtgcganttatctggacttgtcaacc

SEQ ID NO: 59 - DNA, 53 bp, synthetic construct
  misc_feature 1..53: note = Primer sequence
  misc_feature 1..53: note = pr-15976 (attb1_dmd9_f)
  source 1..53: mol_type = other DNA
ggggacaagtttgtacaaaaaagcaggctatggctccatactctagaatctac

SEQ ID NO: 60 - DNA, 64 bp, synthetic construct
  misc_feature 1..64: note = Primer sequence
  misc_feature 1..64: note = pr-15977 (attb2_dmd9_r)
  source 1..64: mol_type = other DNA
ggggaccactttgtacaagaaagctgggtttatctggacttgtcaaccaacaaaacgtttctag

SEQ ID NO: 61 - DNA, 53 bp, synthetic construct
  misc_feature 1..53: note = Primer sequence
  misc_feature 1..53: note = pr-15978 (attb1_phd9_f)
  source 1..53: mol_type = other DNA
ggggacaagtttgtacaaaaaagcaggctatggccctgaagctgaaccccttc

SEQ ID NO: 62 - DNA, 54 bp, synthetic construct
  misc_feature 1..54: note = Primer sequence
  misc_feature 1..54: note = pr-15979 (attb2_phd9_r)
  source 1..54: mol_type = other DNA
ggggaccactttgtacaagaaagctgggtttacagcttcacctgtcggtcgaag

SEQ ID NO: 63 - DNA, 52 bp, synthetic construct
  misc_feature 1..52: note = Primer sequence
  misc_feature 1..52: note = pr-15980 (attb1_rcd9_f)
  source 1..52: mol_type = other DNA
ggggacaagtttgtacaaaaaagcaggctatgggcgtcctgctgaacatctg

SEQ ID NO: 64 - DNA, 53 bp, synthetic construct
  misc_feature 1..53: note = Primer sequence
  misc_feature 1..53: note = pr-15981 (attb1_rcd9_r)
  source 1..53: mol_type = other DNA
ggggaccactttgtacaagaaagctgggtttagacctttcggtcgaagatcca

SEQ ID NO: 65 - protein, 335 aa, Choristoneura rosaceana
MAPNVEDMESDLPESEEKLEKLVAPQAAPRKYQIIYTNLLTFGYWHIAGLYGLYLCFTSAKWQTIILALILNEMAILGITAGAHRLWAHRSYKATVPLQIILIIFNSLSFQNSAIHWIRDHRMHHKYSDTDGDPHNASRGFFYSHVGWLLVKKHPEVKKRAKTIDMSDIYSNPILRFQKKYAIPFIGMICFVLPTIIPMYFWGETLSNAWHITMLRYVFSLNSIFLVNSAAHLYGYRPYDKNILPAENKMTFIACLGENFHNYHHVFPWDYRASELGNIGMNWTAKFIDFFAWIGWAYDLKTASDENIKSRMKRTGDGTDVSGQKYSCESSEVLQ

SEQ ID NO: 66 - protein, 334 aa, Choristoneura parallela
MAPNVEDMESDMPESEKWEKLVAPQAAPRKYEIIYTNLLTFGYGHIAGLYGLYLCFTSAKWQTVILAIILNEMAILGITAGAHRLWSHRSYKAAVPLQIILMIFNSLAFQNSAINWVRDHRMHHKYSDTDGDPHNASRGFFYSHVGWLLVKKHPEVKKRGKMIDMSDIYSNPVLRFQKKYAIPFIGMICFVLPTIIPMYFWGETLSNAWHITMLRYVFSLNSIFLVNSAAHLYGYRPYDKNILPAENKIALIACLGDSFHNYHHVFPWDYRASELGNIGMNWTAQFIDFFAWIGWAYDLKTASDENINSRMKRTGDGTDISGQKYSCESSEVLQ

SEQ ID NO: 67 - DNA, 981 bp, synthetic construct
  misc_feature 1..981: note = Artificial sequence
  source 1..981: mol_type = other DNA
  CDS 1..981: note = codon-optimised for Y. lipolytica
atggtgcccaacaagggttcttccgacgtcctgtctgagcactccgagccccagttcaccaagctgattgctccccaggctggcccccgaaagtacaagatcgtgtaccgaaacctgctgaccttcggatactggcacctgtctgccgtctacggtctgtacctgtgtttcacctgcgccaagtgggctaccattctgttcgccttcttcctgtacgtgatcgctgagatcggcattaccggcggagcccaccgactgtgggctcaccgaacctacaaggccaagctgcccctggagatcctgctgctgattatgaactctatcgctttccaggacaccgccttcacctgggctcgagatcaccgactgcaccacaagtactctgacaccgacgctgaccctcacaacgctacccgaggtttcttctactcccacgtgggctggctgctggtcaagaagcaccccgaggtgaaggcccggggaaagtacctgtccctggacgacctgaagaacaaccccctgctgaagttccagaagaagtacgctatcctggtcattggcaccctgtgtttcctgatgcccaccttcgtgcccgtctacttctggggtgagggcatttctaccgcctggaacatcaacctgctgcgatacgtgatgaacctgaacatgaccttcctggtcaactccgccgctcacattttcggcaacaagccctacgacaagtctattgcctccgtgcagaacatctctgtctccctggctaccttcggagagggtttccacaactaccaccacacctacccttgggactaccgagctgctgagctgggcaacaaccgactgaacatgaccaccgccttcattgacttcttcgcctggatcggatgggcttacgacctgaagtccgtcccccaggaagccatcgctaagcgatgcgctaagaccggcgacggaaccgacatgtggggacgaaagcgatag

SEQ ID NO: 68 - protein, 326 aa, synthetic construct
  REGION 1..326: note = Synthetic Construct
MVPNKGSSDVLSEHSEPQFTKLIAPQAGPRKYKIVYRNLLTFGYWHLSAVYGLYLCFTCAKWATILFAFFLYVIAEIGITGGAHRLWAHRTYKAKLPLEILLLIMNSIAFQDTAFTWARDHRLHHKYSDTDADPHNATRGFFYSHVGWLLVKKHPEVKARGKYLSLDDLKNNPLLKFQKKYAILVIGTLCFLMPTFVPVYFWGEGISTAWNINLLRYVMNLNMTFLVNSAAHIFGNKPYDKSIASVQNISVSLATFGEGFHNYHHTYPWDYRAAELGNNRLNMTTAFIDFFAWIGWAYDLKSVPQEAIAKRCAKTGDGTDMWGRKR

SEQ ID NO: 69 - DNA, 1368 bp, synthetic construct; identical to SEQ ID NO: 43
  misc_feature 1..1368: note = Artificial sequence
  misc_feature 1..1368: note = Y. lipolytica codon-optimized nucleotide sequence of Helicoverpaarmigera fatty acyl reductase
  source 1..1368: mol_type = other DNA

SEQ ID NO: 70 - DNA, 1362 bp, synthetic construct; identical to SEQ ID NO: 32
  misc_feature 1..1362: note = Artificial sequence
  misc_feature 1..1362: note = S. cerevisiae codon-optimized nucleotide sequence of Heliothissubflexa fatty acyl reductase
  source 1..1362: mol_type = other DNA

SEQ ID NO: 71 - protein, 1850 aa, Yarrowia lipolytica
MHPEVEQELAHVLLTELLAYQFASPVRWIETQDVLFKQFNVERVVEVGPSPTLAGMAQRTLKSKYESYDAALSLQREILCYSKDQKDIYYLADEADEAPAPAAGGDAPAAPAAAAPAAAAAPAAAAAPSGPVAKVEDAPVKAQEILHALVAHKLKKTPEQVPLSKAIKDLVGGKSTIQNEILGDLGKEFGATPEKPEDTPLGELAESFQASFDGKLGKQSSSLIARLMSSKMPGGFSLTSARSYLDSRWGLAAGRQDSVLLVALMNEPKNRLGSEAEAKAYLDEQTQKYAASAGLNLSAPAGGAEGGNGGGAVIDSAAFDALTKDQRYLVQQQLELFANYLKQDLRQGSKVAAAQKEAMDILQAELDLWNSEHGEVYAEGIKPAFSALKARVYDSYWNWARQDSLSMYFDIVFGRLSTVDREIMAKCIHLMNRTNHNLIDYMQYHMDHVPVHKGATYELAKQLGLQLLENCKETLTEAPVYKDVSYPTGPQTTIDVKGNIVYNEVPRPNVRKLEQYVHEMACGGELTKDPSFVGEGVQGELKKLYSQISALAKTQTGSTLDIEALYSDLVAKISQAEDASKPVVENKAVSASITPGTLPFLHIKKKTELGAWNYDSETTATYLDGLEVAARDGLTFQGKTALITGAGAGSIGASILQGLISGGCKVIVTTSRYSRKVTEYYQSLYTKFGAKGSTLIVVPFNQGSKKDVDELVSFIYNDPKNGGLGWDLDFVVPFAALPENGIELEHIDSKSELAHRIMLTNLLRLLGNVKKQKVAHSYETRPAQVMLPLSPNHGNFGSDGLYSESKISLETLFNRWHTESWGSYLTIVGVVIGWTRGTGLMSANNITAEGLEQLGVRTFSQTEMAFSIMGLMTKDIVRLAQNSPVWADLNGGFQYIPDLKGVVGKIRRDIVETSEIRRAVAQETAIEQKVVNGPHADLPYQKVEVKPRANLKFDFPTLKSYAEVKELSPAGDALEGLLDLSSVIVVTGFAEVGPWGNARTRWDMEANGVFSLEGAIEMAWIMGLIKHHNGPLPGMPQYSGWIDTKTKQPVDDRDIKTKYEDYLLEHAGIRLIEPELFHGYNPKKKTFLQEVIVEHDLEPFEASKESAEQFALEQGANVEIFAVPESDQWTVRLLKGAKLLIPKALKFDRLVAGQIPTGWDARRYGIPEDICDQVDPITLYALVSTVEALLASGITDPYEFYKYVHVSEVGNCSGSGMGGITALRGMFKDRFMDKPVQNDILQESFINTMSAWVNMLLLSSSGPIKTPVGACATAVESVDIGCETILSGKARICLVGGYDDFQEESSQEFANMNATSNAETEITHGRTPAEMSRPITSTRAGFMEAQGAGTQVLMAADLAIAMGVPIYCIVGYVNTATDKIGRSVPAPGKGILTTAREHQTLKHANPLLNIKYRKRQLDSRLRDIKRWAEGEMEAIDIELDDVSDADKESFIQERSAHIQSQSDRMIREAKNSWGNAFFKQDARISPIRGALATYGLTIDDISVASFHGTSTKANEKNETTTVNAMLEHLGRTRGNPVYGIFQKYLTGHPKGAAGAWMLNGAIQCLNSGIIPGNRNADNVDAYFEQCQHVVFPSRSLQTDGLKAASVTSFGFGQKGAQAIVIHPDYLYAALTPSEYSEYTTRVAQRYKKAYRYYHNAIAEESMFQAKDKAPYSAELEQEVYLDPLVRVHQNEDTEQYSFNAKDLAASAFVKNSHKDTAKVLANLTSQVSGSGKNVGVDVEAISAINIDNDTFLDRNFTANEQAYCFKAPSPQSSFAGTWSAKEAVFKSLGVKSQGGGAELKSIEITRDGNGAPVVVLHGAAKDAAASKGISTVKVSISHDDSQAVAVAVAE

SEQ ID NO: 72 - protein, 334 aa, Yarrowia lipolytica
MKLSTILFTACATLAAALPSPITPSEAAVLQKRVYTSTETSHIDQESYNFFEKYARLANIGYCVGPGTKIFKPFNCGLQCAHFPNVELIEEFHDPRLIFDVSGYLAVDHASKQIYLVIRGTHSLEDVITDIRIMQAPLTNFDLAANISSTATCDDCLVHNGFIQSYNNTYNQIGPKLDSVIEQYPDYQIAVTGHSLGGAAALLFGINLKVNGHDPLVVTLGQPIVGNAGFANWVDKLFFGQENPDVSKVSKDRKLYRITHRGDIVPQVPFWDGYQHCSGEVFIDWPLIHPPLSNVVMCQGQSNKQCSAGNTLLQQVNVIGNHLQYFVTEGVCGI

SEQ ID NO: 73 - protein, 366 aa, Yarrowia lipolytica
MVSFGARIKDFFSVLLFGAASTSSSTKTALVSQGFYDAALDFSHLSNIAYCVNAPITPLKSDFSCGQSCVHFPDIELVHIFGGDFFSTSITGYLALDHVKKEKYVVFRGTFSIADAITDIQFQQSSFLVNVPALNTFIANDTAPEAQIDCKQCKIHDGFSKAFTETWHNIGDLLEQHLDSYPDYQLYVTGHSLGAAMALLGATSIKLRGYDPILINYGQPRVGNKAFADYISALWFGNGDGLEINQQRRLYRMTHWNDVFVGLPNWDGYTHSNGEVYIKGKYVNPPLKDVFSCAGGENSKCYRSEFNLLAQINLLQNHLCYIDYIGFCALNVGRRELNDLPHYNGPYKYGHKTEEQFIAEGLELSN

SEQ ID NO: 74 - protein, 371 aa, Yarrowia lipolytica
MVSLSARIKDFFSVLLLGAATITPSTQTAGVSQGFYDFARDFAHLSNIAYCVNAPITPLNPDFTCGNSCKHFPEIELVKTFGGNFFKTSITGYLAVDHVKKEKYVVFRGTFSLADAITDMQFQLSPFLVDVPALNTFSANDTTAEAQTHCEGCKIHDGFSKAFTETWGNIGEDLQKHLDANPDYQLYVTGHSLGAAMALLGATSIKLKGYDPILINYGQPRVGNKPFAEFINKLWFGEGNGLEITPERKLYRMTHWNDIFVGLPNWEGYTHSNGEVYINNRFINPPLKDVISCAGGENSKCYRSSFSLLSQINLLQNHLAYIDYIGYCALNIGRRELADQEHYTGPYYYGHRSEEDFKKLGLELSTPQVEN